European Patent Specification EP 3 262 065 B1, published April 3, 2024. Title: METHODS AND COMPOSITIONS FOR TREATING DYSTROGLYCANOPATHY DISORDERS. Applicant: THE CHARLOTTE MECKLENBURG HOSPITAL AUTHORITY D/B/A CAROLINAS HEALTHCARE SYSTEM Long Lu, Qi. The sequence listing filed with the application follows.

SEQUENCE LISTING (2 sequences)

SEQ ID NO: 1 - DNA, 1488 bp, Artificial
  Optimized nucleotide coding sequence for FKRP
atgagactgacaagatgccaggccgccctggccgctgccatcacactgaatctgctggtgctgttctatgtgtcctggctgcagcaccagccccggaactctagagccagaggcccaagaagggcctctgccgccggacctagagtgacagtgctcgtgcgcgagttcgaggccttcgacaatgccgtgcccgagctggtggacagcttcctgcagcaagaccctgctcagcctgtggtggtggccgccgatacactgccttatcctccactggccctgcccagaatccccaatgtgcgactggctctgctgcagcccgccctggatagacctgccgccgctagcagacctgagacatacgtggccaccgagttcgtggccctggtgcctgatggcgccagagctgaagctcccggcctgctggaaagaatggtggaagccctgagagccggcagcgccagactggtggctgctcctgtggctaccgccaaccctgccagatgtctggccctgaatgtgtccctgagagagtggaccgccagatacggcgctgcccctgccgctcctagatgtgatgctctggatggcgacgccgtggtgctgctgagagccagggacctgttcaacctgagcgcccctctggccagacctgtgggcacaagcctgtttctgcagacagccctgaggggctgggccgtgcagctgctggatctgacatttgccgctgccagacagcctcctctggccacagcccatgccagatggaaggccgagagagagggcagagccagaagggctgctctgctgagggccctgggcatcagactggtgtcttgggaaggcggcagactcgagtggttcggctgcaacaaagaaaccacccggtgcttcggcaccgtcgtgggcgatacaccagcctacctgtacgaggaaagatggacccccccttgctgcctgcgggccctgagagaaacagccagatatgtcgtgggcgtgctggaagccgctggcgtgcgatattggctggaaggcggatctctgctgggagccgccaggcacggcgacatcatcccttgggactacgacgtggacctgggcatctacctggaagatgtgggcaactgcgagcagctgagaggcgccgaagccggctctgtggtggatgagaggggcttcgtgtgggagaaggccgtggaaggcgacttcttccgggtgcagtacagcgagagcaaccatctgcatgtggacctgtggcccttctacccccggaacggcgtgatgaccaaggacacctggctggaccaccggcaggacgtggaattccccgagcactttctgcagcccctggtgccactgcctttcgccggatttgtggcccaggcccccaacaactaccggcggttcctggaactgaagttcggccctggcgtgatcgagaacccccagtaccctaaccctgccctgctgagcctgaccggcagcggctaa

SEQ ID NO: 2 - DNA, 1488 bp, Homo sapiens
atgcggctcacccgctgccaggctgccctggcggccgccatcaccctcaaccttctggtcctcttctatgtctcgtggctgcagcaccagcctaggaattcccgggcccgggggccccgtcgtgcctctgctgccggcccccgtgtcaccgtcctggtgcgggagttcgaggcatttgacaacgcggtgcccgagctggtagactccttcctgcagcaagacccagcccagcccgtggtggtggcagccgacacgctcccctacccgcccctggccctgccccgcatccccaacgtgcgtctggcgctgctccagcccgccctggaccggccagccgcagcctcgcgcccggagacctacgtggccaccgagtttgtggccctagtacctgatggggcgcgggctgaggcacctggcctgctggagcgcatggtggaggcgctccgcgcaggaagcgcacgtctggtggccgccccggttgccacggccaaccctgccaggtgcctggccctgaacgtcagcctgcgagagtggaccgcccgctatggcgcagcccccgccgcgccccgctgcgacgccctggacggagatgctgtggtgctcctgcgcgcccgcgacctcttcaacctctcggcgcccctggcccggccggtgggcaccagcctctttctgcagaccgcccttcgcggctgggcggtgcagctgctggacttgaccttcgccgcggcgcgccagcccccgctggccacggcccacgcgcgctggaaggctgagcgcgagggacgcgctcggcgggcggcgctgctccgcgcgctgggcatccgcctagtgagctgggaaggcgggcggctggagtggttcggctgcaacaaggagaccacgcgctgcttcggaaccgtggtgggcgacacgcccgcctacctctacgaggagcgctggacgcccccctgctgcctgcgcgcgctgcgcgagaccgcccgctatgtggtgggcgtgctggaggctgcgggcgtgcgctactggctcgagggcggctcactgctgggggccgcccgccacggggacatcatcccatgggactacgacgtggacctgggcatctacttggaggacgtgggcaactgcgagcagctgcggggggcagaggccggctcggtggtggatgagcgcggcttcgtatgggagaaggcggtcgagggcgactttttccgcgtgcagtacagcgaaagcaaccacttgcacgtggacctgtggcccttctacccccgcaatggcgtcatgaccaaggacacgtggctggaccaccggcaggatgtggagtttcccgagcacttcctgcagccgctggtgcccctgccctttgccggcttcgtggcgcaggcgcctaacaactaccgccgcttcctggagctcaagttcgggcccggggtcatcgagaacccccagtaccccaacccggcactgctgagtctgacgggaagcggctga